European Patent Application EP 4 310 180 A1, published January 24, 2024. Title: A MICROORGANISM OF CORYNEBACTERIUM GENUS HAVING ENHANCED L-ARGININE OR L-CITRULLINE PRODUCTIVITY AND A METHOD FOR PRODUCING L-ARGININE OR L-CITRULLINE USING THE SAME. Applicant: DAESANG CORPORATION. Application EP. The sequence listing filed with the application follows.

SEQUENCE LISTING (22 sequences)

SEQ ID NO: 1 - DNA, 885 bp, Corynebacterium sp.
  source 1..885: mol_type = genomic DNA
ttgcagcacttccgcgacaagattgttgtcgtgaaatatggcggaaacgccatggtggatgatgatctcaaggctgcttttgctgccgacatggtcttcttgcgcaccgtgggcgcaaaaccagtggtggtgcacggtggtggacctcagatttctgagatgctaaaccgtgtgggtctccagggcgagttcaagggtggtttccgtgtgaccactcctgaggtcatggacattgtgcgcatggtgctctttggtcaggtcggtcgcgatttagttggtttgatcaactctcatggcccttacgctgtgggaacctccggtgaggatgccggcctgtttaccgcgcagaagcgcatggtcaacatcgatggcgtacccactgatattggtttggtcggagacatcattaatgtcgatgcctcttccttgatggatatcatcgaggccggtcgcattcctgtggtctctacgattgctccaggcgaagacggccagatttacaacattaacgccgataccgcagcaggtgctttggctgcagcgattggtgcagaacgcctgctggttctcaccaatgtggaaggtctgtacaccgattggcctgataagagctcactggtgtccaagatcaaggccaccgagctggaggccattcttccgggacttgattccggcatgattccaaagatggagtcttgcttgaacgcggtgcgtgggggagtaagcgctgctcatgtcattgacggccgcatcgcgcactcggtgttgctggagcttttgaccatgggtggaattggcacgatggtgctgccggatgtttttgatcgggagaattatcctgaaggcaccgtttttagaaaagacgacaaggatggggaactgtaa

SEQ ID NO: 2 - protein, 294 aa, Corynebacterium sp.
MQHFRDKIVVVKYGGNAMVDDDLKAAFAADMVFLRTVGAKPVVVHGGGPQISEMLNRVGLQGEFKGGFRVTTPEVMDIVRMVLFGQVGRDLVGLINSHGPYAVGTSGEDAGLFTAQKRMVNIDGVPTDIGLVGDIINVDASSLMDIIEAGRIPVVSTIAPGEDGQIYNINADTAAGALAAAIGAERLLVLTNVEGLYTDWPDKSSLVSKIKATELEAILPGLDSGMIPKMESCLNAVRGGVSAAHVIDGRIAHSVLLELLTMGGIGTMVLPDVFDRENYPEGTVFRKDDKDGEL

SEQ ID NO: 3 - DNA, 885 bp, synthetic construct
  source 1..885: mol_type = other DNA
ttgcagcacttccgcgacaagattgttgtcgtgaaatatggcggaaacgccatggtggatgatgatctcaaggctgcttttgctgccgacatggtcttcttgcgcaccgtgggcgcaaaaccagtggtggtgcacggtggtggacctcagatttctgagatgctaaaccgtgtgggtctccagggcgagttcaagggtggtttccgtgtgaccactcctgaggtcatggacattgtgcgcatggtgctctttggtcaggtcggtcgcgatttagttggtttgatcaactctcatggcccttacgctgtgggaacctccggtgaggatgccggcctgtttaccgcgcagaagcgcatggtcaacatcgatggcgtacccactgatattggtttggtcggagacatcattaatgtcgatgcctcttccttgatggatatcatcgaggccggtcgcattcctgtggtctctacgattgctccaggcgaagacggccagatttacaacattaacgccgataccgcagcaggtgctttggctgcagcgattggtgcagaacgcctgctggttctcaccaatgtggaaggtctgtacaccgattggcctgataagagctcactggtgtccaagatcaaggccaccgagctggaggccattcttccgggacttgattccggcatgattccaaagatggagtcttgcttgaacgcggtgcgtgggggagtaagcgctgctcatgtcattgacggccgcatcgcgcactcggtgttgctgctgcttttgaccatgggtggaattggcacgatggtgctgccggatgtttttgatcgggagaattatcctgaaggcaccgtttttagaaaagacgacaaggatggggaactgtaa

SEQ ID NO: 4 - protein, 294 aa, synthetic construct
MQHFRDKIVVVKYGGNAMVDDDLKAAFAADMVFLRTVGAKPVVVHGGGPQISEMLNRVGLQGEFKGGFRVTTPEVMDIVRMVLFGQVGRDLVGLINSHGPYAVGTSGEDAGLFTAQKRMVNIDGVPTDIGLVGDIINVDASSLMDIIEAGRIPVVSTIAPGEDGQIYNINADTAAGALAAAIGAERLLVLTNVEGLYTDWPDKSSLVSKIKATELEAILPGLDSGMIPKMESCLNAVRGGVSAAHVIDGRIAHSVLLLLLTMGGIGTMVLPDVFDRENYPEGTVFRKDDKDGEL

SEQ ID NO: 5 - DNA, 885 bp, synthetic construct
  source 1..885: mol_type = other DNA
ttgcagcacttccgcgacaagattgttgtcgtgaaatatggcggaaacgccatggtggatgatgatctcaaggctgcttttgctgccgacatggtcttcttgcgcaccgtgggcgcaaaaccagtggtggtgcacggtggtggacctcagatttctgagatgctaaaccgtgtgggtctccagggcgagttcaagggtggtttccgtgtgaccactcctgaggtcatggacattgtgcgcatggtgctctttggtcaggtcggtcgcgatttagttggtttgatcaactctcatggcccttacgctgtgggaacctccggtgaggatgccggcctgtttaccgcgcagaagcgcatggtcaacatcgatggcgtacccactgatattggtttggtcggagacatcattaatgtcgatgcctcttccttgatggatatcatcgaggccggtcgcattcctgtggtctctacgattgctccaggcgaagacggccagatttacaacattaacgccgataccgcagcaggtgctttggctgcagcgattggtgcagaacgcctgctggttctcaccaatgtggaaggtctgtacaccgattggcctgataagagctcactggtgtccaagatcaaggccaccgagctggaggccattcttccgggacttgattccggcatgattccaaagatggagtcttgcttgaacgcggtgcgtgggggagtaagcgctgctcatgtcattgacggccgcatcgcgcactcggtgttgctggcgcttttgaccatgggtggaattggcacgatggtgctgccggatgtttttgatcgggagaattatcctgaaggcaccgtttttagaaaagacgacaaggatggggaactgtaa

SEQ ID NO: 6 - protein, 294 aa, synthetic construct
MQHFRDKIVVVKYGGNAMVDDDLKAAFAADMVFLRTVGAKPVVVHGGGPQISEMLNRVGLQGEFKGGFRVTTPEVMDIVRMVLFGQVGRDLVGLINSHGPYAVGTSGEDAGLFTAQKRMVNIDGVPTDIGLVGDIINVDASSLMDIIEAGRIPVVSTIAPGEDGQIYNINADTAAGALAAAIGAERLLVLTNVEGLYTDWPDKSSLVSKIKATELEAILPGLDSGMIPKMESCLNAVRGGVSAAHVIDGRIAHSVLLALLTMGGIGTMVLPDVFDRENYPEGTVFRKDDKDGEL

SEQ ID NO: 7 - DNA, 885 bp, synthetic construct
  source 1..885: mol_type = other DNA
ttgcagcacttccgcgacaagattgttgtcgtgaaatatggcggaaacgccatggtggatgatgatctcaaggctgcttttgctgccgacatggtcttcttgcgcaccgtgggcgcaaaaccagtggtggtgcacggtggtggacctcagatttctgagatgctaaaccgtgtgggtctccagggcgagttcaagggtggtttccgtgtgaccactcctgaggtcatggacattgtgcgcatggtgctctttggtcaggtcggtcgcgatttagttggtttgatcaactctcatggcccttacgctgtgggaacctccggtgaggatgccggcctgtttaccgcgcagaagcgcatggtcaacatcgatggcgtacccactgatattggtttggtcggagacatcattaatgtcgatgcctcttccttgatggatatcatcgaggccggtcgcattcctgtggtctctacgattgctccaggcgaagacggccagatttacaacattaacgccgataccgcagcaggtgctttggctgcagcgattggtgcagaacgcctgctggttctcaccaatgtggaaggtctgtacaccgattggcctgataagagctcactggtgtccaagatcaaggccaccgagctggaggccattcttccgggacttgattccggcatgattccaaagatggagtcttgcttgaacgcggtgcgtgggggagtaagcgctgctgatgtcattgacggccgcatcgcgcactcggtgttgctggagcttttgaccatgggtggaattggcacgatggtgctgccggatgtttttgatcgggagaattatcctgaaggcaccgtttttagaaaagacgacaaggatggggaactgtaa

SEQ ID NO: 8 - protein, 294 aa, synthetic construct
MQHFRDKIVVVKYGGNAMVDDDLKAAFAADMVFLRTVGAKPVVVHGGGPQISEMLNRVGLQGEFKGGFRVTTPEVMDIVRMVLFGQVGRDLVGLINSHGPYAVGTSGEDAGLFTAQKRMVNIDGVPTDIGLVGDIINVDASSLMDIIEAGRIPVVSTIAPGEDGQIYNINADTAAGALAAAIGAERLLVLTNVEGLYTDWPDKSSLVSKIKATELEAILPGLDSGMIPKMESCLNAVRGGVSAADVIDGRIAHSVLLELLTMGGIGTMVLPDVFDRENYPEGTVFRKDDKDGEL

SEQ ID NO: 9 - DNA, 33 bp, synthetic construct
  source 1..33: mol_type = other DNA
tgattacgccactgacacggtggataaggaaac

SEQ ID NO: 10 - DNA, 23 bp, synthetic construct
  source 1..23: mol_type = other DNA
actgacacggtggataaggaaac

SEQ ID NO: 11 - DNA, 18 bp, synthetic construct
  source 1..18: mol_type = other DNA
agcagcaacaccgagtgc

SEQ ID NO: 12 - DNA, 20 bp, synthetic construct
  source 1..20: mol_type = other DNA
ggtcaaaagcagcagcaaca

SEQ ID NO: 13 - DNA, 28 bp, synthetic construct
  source 1..28: mol_type = other DNA
gcttttgaccatgggtggaattggcacg

SEQ ID NO: 14 - DNA, 18 bp, synthetic construct
  source 1..18: mol_type = other DNA
atgggtggaattggcacg

SEQ ID NO: 15 - DNA, 18 bp, synthetic construct
  source 1..18: mol_type = other DNA
catcgggaacaacgccat

SEQ ID NO: 16 - DNA, 19 bp, synthetic construct
  source 1..19: mol_type = other DNA
atggtcaccacatcgggaa

SEQ ID NO: 17 - DNA, 16 bp, synthetic construct
  source 1..16: mol_type = other DNA
gccagcaacaccgagt

SEQ ID NO: 18 - DNA, 20 bp, synthetic construct
  source 1..20: mol_type = other DNA
ggtcaaaagcgccagcaaca

SEQ ID NO: 19 - DNA, 21 bp, synthetic construct
  source 1..21: mol_type = other DNA
caatgacatcagcagcgctta

SEQ ID NO: 20 - DNA, 17 bp, synthetic construct
  source 1..17: mol_type = other DNA
atgcggccgtcaatgac

SEQ ID NO: 21 - DNA, 28 bp, synthetic construct
  source 1..28: mol_type = other DNA
acggccgcatcgcgcactcggtgttgct

SEQ ID NO: 22 - DNA, 18 bp, synthetic construct
  source 1..18: mol_type = other DNA
cgcgcactcggtgttgct